European Patent Application EP 4 650 366 A1, published November 19, 2025. Title: TGFβ1 BINDING MOLECULE, GARP-TGFβ1 BINDING MOLECULE AND MEDICAL USE THEREOF. Applicant: BEIJING TUO JIE BIOPHARMACEUTICAL CO. LTD. Application WO PCT/CN2024/071321, filed January 9, 2024. The sequence listing filed with the application follows.

SEQUENCE LISTING (126 sequences)

SEQ ID NO: 1 - protein, 390 aa, Homo sapiens
MPPSGLRLLLLLLPLLWLLVLTPGRPAAGLSTCKTIDMELVKRKRIEAIRGQILSKLRLASPPSQGEVPPGPLPEAVLALYNSTRDRVAGESAEPEPEPEADYYAKEVTRVLMVETHNEIYDKFKQSTHSIYMFFNTSELREAVPEPVLLSRAELRLLRLKLKVEQHVELYQKYSNNSWRYLSNRLLAPSDSPEWLSFDVTGVVRQWLSRGGEIEGFRLSAHCSCDSRDNTLQVDINGFTTGRRGDLATIHGMNRPFLLLMATPLERAQHLQSSRHRRALDTNYCFSSTEKNCCVRQLYIDFRKDLGWKWIHEPKGYHANFCLGPCPYIWSLDTQYSKVLALYNQHNPGASAAPCCVPQALEPLPIVYYVGRKPKVEQLSNMIVRSCKCS

SEQ ID NO: 2 - protein, 662 aa, Homo sapiens
MRPQILLLLALLTLGLAAQHQDKVPCKMVDKKVSCQVLGLLQVPSVLPPDTETLDLSGNQLRSILASPLGFYTALRHLDLSTNEISFLQPGAFQALTHLEHLSLAHNRLAMATALSAGGLGPLPRVTSLDLSGNSLYSGLLERLLGEAPSLHTLSLAENSLTRLTRHTFRDMPALEQLDLHSNVLMDIEDGAFEGLPRLTHLNLSRNSLTCISDFSLQQLRVLDLSCNSIEAFQTASQPQAEFQLTWLDLRENKLLHFPDLAALPRLIYLNLSNNLIRLPTGPPQDSKGIHAPSEGWSALPLSAPSGNASGRPLSQLLNLDLSYNEIELIPDSFLEHLTSLCFLNLSRNCLRTFEARRLGSLPCLMLLDLSHNALETLELGARALGSLRTLLLQGNALRDLPPYTFANLASLQRLNLQGNRVSPCGGPDEPGPSGCVAFSGITSLRSLSLVDNEIELLRAGAFLHTPLTELDLSSNPGLEVATGALGGLEASLEVLALQGNGLMVLQVDLPCFICLKRLNLAENRLSHLPAWTQAVSLEVLDLRNNSFSLLPGSAMGGLETSLRRLYLQGNPLSCCGNGWLAAQLHQGRVDVDATQDLICRFSSQEEVSLSHVRPEDCEKGGLKNINLIIILTFILVSAILLTTLAACCCVRRQKFNQQYKA

SEQ ID NO: 3 - protein, 390 aa, Mus musculus
MPPSGLRLLPLLLPLPWLLVLTPGRPAAGLSTCKTIDMELVKRKRIEAIRGQILSKLRLASPPSQGEVPPGPLPEAVLALYNSTRDRVAGESADPEPEPEADYYAKEVTRVLMVDRNNAIYEKTKDISHSIYMFFNTSDIREAVPEPPLLSRAELRLQRLKSSVEQHVELYQKYSNNSWRYLGNRLLTPTDTPEWLSFDVTGVVRQWLNQGDGIQGFRFSAHCSCDSKDNKLHVEINGISPKRRGDLGTIHDMNRPFLLLMATPLERAQHLHSSRHRRALDTNYCFSSTEKNCCVRQLYIDFRKDLGWKWIHEPKGYHANFCLGPCPYIWSLDTQYSKVLALYNQHNPGASASPCCVPQALEPLPIVYYVGRKPKVEQLSNMIVRSCKCS

SEQ ID NO: 4 - protein, 663 aa, Mus musculus
MSHQILLLLAMLTLGLAISQRREQVPCRTVNKEALCHGLGLLQVPSVLSLDIQALYLSGNQLQSILVSPLGFYTALRHLDLSDNQISFLQAGVFQALPYLEHLNLAHNRLATGMALNSGGLGRLPLLVSLDLSGNSLHGNLVERLLGETPRLRTLSLAENSLTRLARHTFWGMPAVEQLDLHSNVLMDIEDGAFEALPHLTHLNLSRNSLTCISDFSLQQLQVLDLSCNSIEAFQTAPEPQAQFQLAWLDLRENKLLHFPDLAVFPRLIYLNVSNNLIQLPAGLPRGSEDLHAPSEGWSASPLSNPSRNASTHPLSQLLNLDLSYNEIELVPASFLEHLTSLRFLNLSRNCLRSFEARQVDSLPCLVLLDLSHNVLEALELGTKVLGSLQTLLLQDNALQELPPYTFASLASLQRLNLQGNQVSPCGGPAEPGPPGCVDFSGIPTLHVLNMAGNSMGMLRAGSFLHTPLTELDLSTNPGLDVATGALVGLEASLEVLELQGNGLTVLRVDLPCFLRLKRLNLAENQLSHLPAWTRAVSLEVLDLRNNSFSLLPGNAMGGLETSLRRLYLQGNPLSCCGNGWLAAQLHQGRVDVDATQDLICRFGSQEELSLSLVRPEDCEKGGLKNVNLILLLSFTLVSAIVLTTLATICFLRRQKLSQQYKA

SEQ ID NO: 5 - protein, 651 aa, synthetic construct
  source 1..651: note = GARP-avi-his
HQDKVPCKMVDKKVSCQVLGLLQVPSVLPPDTETLDLSGNQLRSILASPLGFYTALRHLDLSTNEISFLQPGAFQALTHLEHLSLAHNRLAMATALSAGGLGPLPRVTSLDLSGNSLYSGLLERLLGEAPSLHTLSLAENSLTRLTRHTFRDMPALEQLDLHSNVLMDIEDGAFEGLPRLTHLNLSRNSLTCISDFSLQQLRVLDLSCNSIEAFQTASQPQAEFQLTWLDLRENKLLHFPDLAALPRLIYLNLSNNLIRLPTGPPQDSKGIHAPSEGWSALPLSAPSGNASGRPLSQLLNLDLSYNEIELIPDSFLEHLTSLCFLNLSRNCLRTFEARRLGSLPCLMLLDLSHNALETLELGARALGSLRTLLLQGNALRDLPPYTFANLASLQRLNLQGNRVSPCGGPDEPGPSGCVAFSGITSLRSLSLVDNEIELLRAGAFLHTPLTELDLSSNPGLEVATGALGGLEASLEVLALQGNGLMVLQVDLPCFICLKRLNLAENRLSHLPAWTQAVSLEVLDLRNNSFSLLPGSAMGGLETSLRRLYLQGNPLSCCGNGWLAAQLHQGRVDVDATQDLICRFSSQEEVSLSHVRPEDCEKGGLKNINGGGGSGGGGSGLNDIFEAQKIEWHEGGGGSGGGGSHHHHHHHH

SEQ ID NO: 6 - protein, 361 aa, Homo sapiens
LSTCKTIDMELVKRKRIEAIRGQILSKLRLASPPSQGEVPPGPLPEAVLALYNSTRDRVAGESAEPEPEPEADYYAKEVTRVLMVETHNEIYDKFKQSTHSIYMFFNTSELREAVPEPVLLSRAELRLLRLKLKVEQHVELYQKYSNNSWRYLSNRLLAPSDSPEWLSFDVTGVVRQWLSRGGEIEGFRLSAHCSCDSRDNTLQVDINGFTTGRRGDLATIHGMNRPFLLLMATPLERAQHLQSSRHRRALDTNYCFSSTEKNCCVRQLYIDFRKDLGWKWIHEPKGYHANFCLGPCPYIWSLDTQYSKVLALYNQHNPGASAAPCCVPQALEPLPIVYYVGRKPKVEQLSNMIVRSCKCS

SEQ ID NO: 7 - protein, 404 aa, synthetic construct
  source 1..404: note; note (original language) = TGFβ1 C4S
HHHHHHHHGGGGSGGGGSGLNDIFEAQKIEWHEGGGGSGGGGSLSTSKTIDMELVKRKRIEAIRGQILSKLRLASPPSQGEVPPGPLPEAVLALYNSTRDRVAGESAEPEPEPEADYYAKEVTRVLMVETHNEIYDKFKQSTHSIYMFFNTSELREAVPEPVLLSRAELRLLRLKLKVEQHVELYQKYSNNSWRYLSNRLLAPSDSPEWLSFDVTGVVRQWLSRGGEIEGFRLSAHCSCDSRDNTLQVDINGFTTGRRGDLATIHGMNRPFLLLMATPLERAQHLQSSRHRRALDTNYCFSSTEKNCCVRQLYIDFRKDLGWKWIHEPKGYHANFCLGPCPYIWSLDTQYSKVLALYNQHNPGASAAPCCVPQALEPLPIVYYVGRKPKVEQLSNMIVRSCKCS

SEQ ID NO: 8 - protein, 654 aa, synthetic construct
  source 1..654: note = GARP-avi-his
ISQRREQVPCRTVNKEALCHGLGLLQVPSVLSLDIQALYLSGNQLQSILVSPLGFYTALRHLDLSDNQISFLQAGVFQALPYLEHLNLAHNRLATGMALNSGGLGRLPLLVSLDLSGNSLHGNLVERLLGETPRLRTLSLAENSLTRLARHTFWGMPAVEQLDLHSNVLMDIEDGAFEALPHLTHLNLSRNSLTCISDFSLQQLQVLDLSCNSIEAFQTAPEPQAQFQLAWLDLRENKLLHFPDLAVFPRLIYLNVSNNLIQLPAGLPRGSEDLHAPSEGWSASPLSNPSRNASTHPLSQLLNLDLSYNEIELVPASFLEHLTSLRFLNLSRNCLRSFEARQVDSLPCLVLLDLSHNVLEALELGTKVLGSLQTLLLQDNALQELPPYTFASLASLQRLNLQGNQVSPCGGPAEPGPPGCVDFSGIPTLHVLNMAGNSMGMLRAGSFLHTPLTELDLSTNPGLDVATGALVGLEASLEVLELQGNGLTVLRVDLPCFLRLKRLNLAENQLSHLPAWTRAVSLEVLDLRNNSFSLLPGNAMGGLETSLRRLYLQGNPLSCCGNGWLAAQLHQGRVDVDATQDLICRFGSQEELSLSLVRPEDCEKGGLKNVNGGGGSGGGGSGLNDIFEAQKIEWHEGGGGSGGGGSHHHHHHHH

SEQ ID NO: 9 - protein, 361 aa, Mus musculus
LSTCKTIDMELVKRKRIEAIRGQILSKLRLASPPSQGEVPPGPLPEAVLALYNSTRDRVAGESADPEPEPEADYYAKEVTRVLMVDRNNAIYEKTKDISHSIYMFFNTSDIREAVPEPPLLSRAELRLQRLKSSVEQHVELYQKYSNNSWRYLGNRLLTPTDTPEWLSFDVTGVVRQWLNQGDGIQGFRFSAHCSCDSKDNKLHVEINGISPKRRGDLGTIHDMNRPFLLLMATPLERAQHLHSSRHRRALDTNYCFSSTEKNCCVRQLYIDFRKDLGWKWIHEPKGYHANFCLGPCPYIWSLDTQYSKVLALYNQHNPGASASPCCVPQALEPLPIVYYVGRKPKVEQLSNMIVRSCKCS

SEQ ID NO: 10 - protein, 404 aa, synthetic construct
  source 1..404: note; note (original language) = TGFβ1 C4S
HHHHHHHHGGGGSGGGGSGLNDIFEAQKIEWHEGGGGSGGGGSLSTSKTIDMELVKRKRIEAIRGQILSKLRLASPPSQGEVPPGPLPEAVLALYNSTRDRVAGESADPEPEPEADYYAKEVTRVLMVDRNNAIYEKTKDISHSIYMFFNTSDIREAVPEPPLLSRAELRLQRLKSSVEQHVELYQKYSNNSWRYLGNRLLTPTDTPEWLSFDVTGVVRQWLNQGDGIQGFRFSAHCSCDSKDNKLHVEINGISPKRRGDLGTIHDMNRPFLLLMATPLERAQHLHSSRHRRALDTNYCFSSTEKNCCVRQLYIDFRKDLGWKWIHEPKGYHANFCLGPCPYIWSLDTQYSKVLALYNQHNPGASASPCCVPQALEPLPIVYYVGRKPKVEQLSNMIVRSCKCS

SEQ ID NO: 11 - protein, 121 aa, synthetic construct
  source 1..121: note = H27 VH
EVQLLESGGGLVQPGGSLRLSCAASGFTFSSYAMSWVRQAPGKGLEWVSAISGSGGSTYYADSVKGRFTISRDNSKNTLYLQMNSLRAEDTAVYYCARVDSSGGYWYFDLWGRGTLVTVSS

SEQ ID NO: 12 - protein, 107 aa, synthetic construct
  source 1..107: note = H27 VL
DIQMTQSPSSLSASVGDRVTITCRASQSISSYLNWYQQKPGKAPKLLIYAASSLQSGVPSRFSGSGSGTDFTLTISSLQPEDFATYYCQQSYSTPLTFGGGTKLEIK

SEQ ID NO: 13 - protein, 5 aa, synthetic construct
  source 1..5: note = HCDR1
SYAMS

SEQ ID NO: 14 - protein, 17 aa, synthetic construct
  source 1..17: note = HCDR2
AISGSGGSTYYADSVKG

SEQ ID NO: 15 - protein, 12 aa, synthetic construct
  source 1..12: note = HCDR3
VDSSGGYWYFDL

SEQ ID NO: 16 - protein, 11 aa, synthetic construct
  source 1..11: note = LCDR1
RASQSISSYLN

SEQ ID NO: 17 - protein, 7 aa, synthetic construct
  source 1..7: note = LCDR2
AASSLQS

SEQ ID NO: 18 - protein, 9 aa, synthetic construct
  source 1..9: note = LCDR3
QQSYSTPLT

SEQ ID NO: 19 - protein, 107 aa, synthetic construct [sequence omitted]

SEQ ID NO: 20 - protein, 327 aa, synthetic construct
  source 1..327: note; note (original language) = Human IgG4-S228P heavy chain constant region
ASTKGPSVFPLAPCSRSTSESTAALGCLVKDYFPEPVTVSWNSGALTSGVHTFPAVLQSSGLYSLSSVVTVPSSSLGTKTYTCNVDHKPSNTKVDKRVESKYGPPCPPCPAPEFLGGPSVFLFPPKPKDTLMISRTPEVTCVVVDVSQEDPEVQFNWYVDGVEVHNAKTKPREEQFNSTYRVVSVLTVLHQDWLNGKEYKCKVSNKGLPSSIEKTISKAKGQPREPQVYTLPPSQEEMTKNQVSLTCLVKGFYPSDIAVEWESNGQPENNYKTTPPVLDSDGSFFLYSRLTVDKSRWQEGNVFSCSVMHEALHNHYTQKSLSLSLGK

SEQ ID NO: 21 - protein, 107 aa, synthetic construct
  source 1..107: note = SL2-1
DIQMTQSPSSLSASVGDRVTITCRASQAISDYLNWYQQKPGKAPKLLIYTASYLTSGVPSRFSGSGSGTDFTLTISSLQPEDFATYYCQQSYSTPLTFGGGTKLEIK

SEQ ID NO: 22 - protein, 107 aa, synthetic construct
  source 1..107: note = SL2-2
DIQMTQSPSSLSASVGDRVTITCRASQFISDYLNWYQQKPGKAPKLLIYTASYLDSGVPSRFSGSGSGTDFTLTISSLQPEDFATYYCQQSYSTPLTFGGGTKLEIK

SEQ ID NO: 23 - protein, 107 aa, synthetic construct
  source 1..107: note = SL2-3
DIQMTQSPSSLSASVGDRVTITCRASQGISEYLNWYQQKPGKAPKLLIYTASYLDSGVPSRFSGSGSGTDFTLTISSLQPEDFATYYCQQSYSTPLTFGGGTKLEIK

SEQ ID NO: 24 - protein, 107 aa, synthetic construct
  source 1..107: note = SL2-4
DIQMTQSPSSLSASVGDRVTITCRASQIISDYLNWYQQKPGKAPKLLIYSASYLESGVPSRFSGSGSGTDFTLTISSLQPEDFATYYCQQSYSTPLTFGGGTKLEIK

SEQ ID NO: 25 - protein, 107 aa, synthetic construct
  source 1..107: note = SL2-5
DIQMTQSPSSLSASVGDRVTITCRASQPISDYLNWYQQKPGKAPKLLIYTASYLESGVPSRFSGSGSGTDFTLTISSLQPEDFATYYCQQSYSTPLTFGGGTKLEIK

SEQ ID NO: 26 - protein, 107 aa, synthetic construct
  source 1..107: note = SL2-6 VL
DIQMTQSPSSLSASVGDRVTITCRASQYISDYLNWYQQKPGKAPKLLIYMASALDSGVPSRFSGSGSGTDFTLTISSLQPEDFATYYCQQSYSTPLTFGGGTKLEIK

SEQ ID NO: 27 - protein, 107 aa, synthetic construct
  source 1..107: note = SL2-8
DIQMTQSPSSLSASVGDRVTITCRASQYISDYLNWYQQKPGKAPKLLIYAASYLESGVPSRFSGSGSGTDFTLTISSLQPEDFATYYCQQSYSTPLTFGGGTKLEIK

SEQ ID NO: 28 - protein, 107 aa, synthetic construct
  source 1..107: note = SL2-9
DIQMTQSPSSLSASVGDRVTITCRASQFISPYLNWYQQKPGKAPKLLIYAASELESGVPSRFSGSGSGTDFTLTISSLQPEDFATYYCQQSYSTPLTFGGGTKLEIK

SEQ ID NO: 29 - protein, 107 aa, synthetic construct
  source 1..107: note = SL2-12
DIQMTQSPSSLSASVGDRVTITCRASQYISDYLNWYQQKPGKAPKLLIYSASYLDSGVPSRFSGSGSGTDFTLTISSLQPEDFATYYCQQSYSTPLTFGGGTKLEIK

SEQ ID NO: 30 - protein, 107 aa, synthetic construct
  source 1..107: note = SL2-13
DIQMTQSPSSLSASVGDRVTITCRASQVISDYLNWYQQKPGKAPKLLIYAASYLDSGVPSRFSGSGSGTDFTLTISSLQPEDFATYYCQQSYSTPLTFGGGTKLEIK

SEQ ID NO: 31 - protein, 107 aa, synthetic construct
  source 1..107: note = SL2-15
DIQMTQSPSSLSASVGDRVTITCRASQKISDYLNWYQQKPGKAPKLLIYAASGLESGVPSRFSGSGSGTDFTLTISSLQPEDFATYYCQQSYSTPLTFGGGTKLEIK

SEQ ID NO: 32 - protein, 107 aa, synthetic construct
  source 1..107: note = SL2-17
DIQMTQSPSSLSASVGDRVTITCRASQGISHYLNWYQQKPGKAPKLLIYAASYLDSGVPSRFSGSGSGTDFTLTISSLQPEDFATYYCQQSYSTPLTFGGGTKLEIK

SEQ ID NO: 33 - protein, 107 aa, synthetic construct
  source 1..107: note = SL2-18
DIQMTQSPSSLSASVGDRVTITCRASQSISEYLNWYQQKPGKAPKLLIYTASYLESGVPSRFSGSGSGTDFTLTISSLQPEDFATYYCQQSYSTPLTFGGGTKLEIK

SEQ ID NO: 34 - protein, 107 aa, synthetic construct
  source 1..107: note = SL2-19
DIQMTQSPSSLSASVGDRVTITCRASQAISPYLNWYQQKPGKAPKLLIYAASELESGVPSRFSGSGSGTDFTLTISSLQPEDFATYYCQQSYSTPLTFGGGTKLEIK

SEQ ID NO: 35 - protein, 107 aa, synthetic construct
  source 1..107: note = SL2-22
DIQMTQSPSSLSASVGDRVTITCRASQSISDYLNWYQQKPGKAPKLLIYTASYLDSGVPSRFSGSGSGTDFTLTISSLQPEDFATYYCQQSYSTPLTFGGGTKLEIK

SEQ ID NO: 36 - protein, 11 aa, synthetic construct
  source 1..11: note = SL2-1 LCDR1
RASQAISDYLN

SEQ ID NO: 37 - protein, 7 aa, synthetic construct
  source 1..7: note = SL2-1 LCDR2
TASYLTS

SEQ ID NO: 38 - protein, 11 aa, synthetic construct
  source 1..11: note = LCDR1
  VARIANT 5: note; note (original language) = X is selected from the group consisting of S, A, F, G, I, P, Y, V, and K
  VARIANT 8: note; note (original language) = X is selected from the group consisting of S, D, E, P, and H
RASQXISXYLN

SEQ ID NO: 39 - protein, 11 aa, synthetic construct
  source 1..11: note = SL2-2 LCDR1
RASQFISDYLN

SEQ ID NO: 40 - protein, 7 aa, synthetic construct
  source 1..7: note = SL2-2 LCDR2
TASYLDS

SEQ ID NO: 41 - protein, 11 aa, synthetic construct
  source 1..11: note = SL2-3 LCDR1
RASQGISEYLN

SEQ ID NO: 42 - protein, 11 aa, synthetic construct
  source 1..11: note = SL2-4 LCDR1
RASQIISDYLN

SEQ ID NO: 43 - protein, 7 aa, synthetic construct
  source 1..7: note = SL2-4 LCDR2
SASYLES

SEQ ID NO: 44 - protein, 11 aa, synthetic construct
  source 1..11: note = SL2-5 LCDR1
RASQPISDYLN

SEQ ID NO: 45 - protein, 7 aa, synthetic construct
  source 1..7: note = SL2-5 LCDR2
TASYLES

SEQ ID NO: 46 - protein, 11 aa, synthetic construct
  source 1..11: note = SL2-6 LCDR1
RASQYISDYLN

SEQ ID NO: 47 - protein, 7 aa, synthetic construct
  source 1..7: note = SL2-6 LCDR2
MASALDS

SEQ ID NO: 48 - protein, 7 aa, synthetic construct
  source 1..7: note = SL2-8 LCDR2
AASYLES

SEQ ID NO: 49 - protein, 11 aa, synthetic construct
  source 1..11: note = SL2-9 LCDR1
RASQFISPYLN

SEQ ID NO: 50 - protein, 7 aa, synthetic construct
  source 1..7: note = SL2-9 LCDR2
AASELES

SEQ ID NO: 51 - protein, 7 aa, synthetic construct
  source 1..7: note = SL2-12 LCDR2
SASYLDS

SEQ ID NO: 52 - protein, 11 aa, synthetic construct
  source 1..11: note = SL2-13 LCDR1
RASQVISDYLN

SEQ ID NO: 53 - protein, 7 aa, synthetic construct
  source 1..7: note = SL2-13 LCDR1
AASYLDS

SEQ ID NO: 54 - protein, 11 aa, synthetic construct
  source 1..11: note = SL2-15 LCDR1
RASQKISDYLN

SEQ ID NO: 55 - protein, 7 aa, synthetic construct
  source 1..7: note = SL2-15 LCDR2
AASGLES

SEQ ID NO: 56 - protein, 11 aa, synthetic construct
  source 1..11: note = SL2-17 LCDR1
RASQGISHYLN

SEQ ID NO: 57 - protein, 11 aa, synthetic construct
  source 1..11: note = SL2-18 LCDR1
RASQSISEYLN

SEQ ID NO: 58 - protein, 11 aa, synthetic construct
  source 1..11: note = SL2-19 LCDR1
RASQAISPYLN

SEQ ID NO: 59 - protein, 11 aa, synthetic construct
  source 1..11: note = SL2-22 LCDR1
RASQSISDYLN

SEQ ID NO: 60 - protein, 447 aa, synthetic construct
  source 1..447: note; note (original language) = Ab6 antibody heavy chain
EVQLVESGGGLVQPGGSLRLSCTASGFTFSSFSMDWVRQAPGKGLEWVSYISPSADTIYYADSVKGRFTISRDNAKNTLYLQMNSLRAEDTAVYYCARGVLDYGDMLMPWGQGTLVTVSSASTKGPSVFPLAPCSRSTSESTAALGCLVKDYFPEPVTVSWNSGALTSGVHTFPAVLQSSGLYSLSSVVTVPSSSLGTKTYTCNVDHKPSNTKVDKRVESKYGPPCPPCPAPEFLGGPSVFLFPPKPKDTLMISRTPEVTCVVVDVSQEDPEVQFNWYVDGVEVHNAKTKPREEQFNSTYRVVSVLTVLHQDWLNGKEYKCKVSNKGLPSSIEKTISKAKGQPREPQVYTLPPSQEEMTKNQVSLTCLVKGFYPSDIAVEWESNGQPENNYKTTPPVLDSDGSFFLYSRLTVDKSRWQEGNVFSCSVMHEALHNHYTQKSLSLSLGK

SEQ ID NO: 61 - protein, 215 aa, synthetic construct
  source 1..215: note; note (original language) = Ab6 antibody light chain
DIQMTQSPSSLSASVGDRVTITCQASQDITNYLNWYQQKPGKAPKLLIYDASNLETGVPSRFSGSGSGTDFTFTISSLQPEDIATYYCQQADNHPPWTFGGGTKVEIKRTVAAPSVFIFPPSDEQLKSGTASVVCLLNNFYPREAKVQWKVDNALQSGNSQESVTEQDSKDSTYSLSSTLTLSKADYEKHKVYACEVTHQGLSSPVTKSFNRGEC

SEQ ID NO: 62 - protein, 452 aa, synthetic construct
  source 1..452: note; note (original language) = Abbv-151 antibody heavy chain
QVQLVQPGAEVRKPGASVKVSCKASGYRFTSYYIDWVRQAPGQGLEWMGRIDPEDAGTKYAQKFQGRVTMTADTSTSTVYVELSSLRSEDTAVYYCARYEWETVVVGDLMYEYEYWGQGTLVTVSSASTKGPSVFPLAPCSRSTSESTAALGCLVKDYFPEPVTVSWNSGALTSGVHTFPAVLQSSGLYSLSSVVTVPSSSLGTKTYTCNVDHKPSNTKVDKRVESKYGPPCPPCPAPEFLGGPSVFLFPPKPKDTLMISRTPEVTCVVVDVSQEDPEVQFNWYVDGVEVHNAKTKPREEQFNSTYRVVSVLTVLHQDWLNGKEYKCKVSNKGLPSSIEKTISKAKGQPREPQVYTLPPSQEEMTKNQVSLTCLVKGFYPSDIAVEWESNGQPENNYKTTPPVLDSDGSFFLYSRLTVDKSRWQEGNVFSCSVMHEALHNHYTQKSLSLSLG

SEQ ID NO: 63 - protein, 214 aa, synthetic construct
  source 1..214: note; note (original language) = Abbv-151 antibody light chain
DIQMTQSPSSLSASVGDRVTITCQASQSISSYLAWYQQKPGQAPKILIYGASRLKTGVPSRFSGSGSGTSFTLTISSLEPEDAATYYCQQYASVPVTFGQGTKVEIKRTVAAPSVFIFPPSDEQLKSGTASVVCLLNNFYPREAKVQWKVDNALQSGNSQESVTEQDSKDSTYSLSSTLTLSKADYEKHKVYACEVTHQGLSSPVTKSFNRGEC

SEQ ID NO: 64 - protein, 7 aa, synthetic construct
  source 1..7: note = LCDR2
  VARIANT 1: note; note (original language) = X is selected from the group consisting of A, T, S, and M
  VARIANT 4: note; note (original language) = X is selected from the group consisting of S, Y, A, E, and G
  VARIANT 6: note; note (original language) = X is selected from the group consisting of Q, T, D, and E
XASXLXS

SEQ ID NO: 65 - protein, 214 aa, synthetic construct
  source 1..214: note; note (original language) = H27 light chain
DIQMTQSPSSLSASVGDRVTITCRASQSISSYLNWYQQKPGKAPKLLIYAASSLQSGVPSRFSGSGSGTDFTLTISSLQPEDFATYYCQQSYSTPLTFGGGTKLEIKRTVAAPSVFIFPPSDEQLKSGTASVVCLLNNFYPREAKVQWKVDNALQSGNSQESVTEQDSKDSTYSLSSTLTLSKADYEKHKVYACEVTHQGLSSPVTKSFNRGEC

SEQ ID NO: 66 - protein, 448 aa, synthetic construct
  source 1..448: note; note (original language) = H27 heavy chain
EVQLLESGGGLVQPGGSLRLSCAASGFTFSSYAMSWVRQAPGKGLEWVSAISGSGGSTYYADSVKGRFTISRDNSKNTLYLQMNSLRAEDTAVYYCARVDSSGGYWYFDLWGRGTLVTVSSASTKGPSVFPLAPCSRSTSESTAALGCLVKDYFPEPVTVSWNSGALTSGVHTFPAVLQSSGLYSLSSVVTVPSSSLGTKTYTCNVDHKPSNTKVDKRVESKYGPPCPPCPAPEFLGGPSVFLFPPKPKDTLMISRTPEVTCVVVDVSQEDPEVQFNWYVDGVEVHNAKTKPREEQFNSTYRVVSVLTVLHQDWLNGKEYKCKVSNKGLPSSIEKTISKAKGQPREPQVYTLPPSQEEMTKNQVSLTCLVKGFYPSDIAVEWESNGQPENNYKTTPPVLDSDGSFFLYSRLTVDKSRWQEGNVFSCSVMHEALHNHYTQKSLSLSLGK

SEQ ID NO: 67 - protein, 214 aa, synthetic construct
  source 1..214: note; note (original language) = SL2-1 light chain LC
DIQMTQSPSSLSASVGDRVTITCRASQAISDYLNWYQQKPGKAPKLLIYTASYLTSGVPSRFSGSGSGTDFTLTISSLQPEDFATYYCQQSYSTPLTFGGGTKLEIKRTVAAPSVFIFPPSDEQLKSGTASVVCLLNNFYPREAKVQWKVDNALQSGNSQESVTEQDSKDSTYSLSSTLTLSKADYEKHKVYACEVTHQGLSSPVTKSFNRGEC

SEQ ID NO: 68 - protein, 214 aa, synthetic construct
  source 1..214: note; note (original language) = SL2-2 light chain LC
DIQMTQSPSSLSASVGDRVTITCRASQFISDYLNWYQQKPGKAPKLLIYTASYLDSGVPSRFSGSGSGTDFTLTISSLQPEDFATYYCQQSYSTPLTFGGGTKLEIKRTVAAPSVFIFPPSDEQLKSGTASVVCLLNNFYPREAKVQWKVDNALQSGNSQESVTEQDSKDSTYSLSSTLTLSKADYEKHKVYACEVTHQGLSSPVTKSFNRGEC

SEQ ID NO: 69 - protein, 214 aa, synthetic construct
  source 1..214: note; note (original language) = SL2-3 light chain LC
DIQMTQSPSSLSASVGDRVTITCRASQGISEYLNWYQQKPGKAPKLLIYTASYLDSGVPSRFSGSGSGTDFTLTISSLQPEDFATYYCQQSYSTPLTFGGGTKLEIKRTVAAPSVFIFPPSDEQLKSGTASVVCLLNNFYPREAKVQWKVDNALQSGNSQESVTEQDSKDSTYSLSSTLTLSKADYEKHKVYACEVTHQGLSSPVTKSFNRGEC

SEQ ID NO: 70 - protein, 214 aa, synthetic construct
  source 1..214: note; note (original language) = SL2-4 light chain LC
DIQMTQSPSSLSASVGDRVTITCRASQIISDYLNWYQQKPGKAPKLLIYSASYLESGVPSRFSGSGSGTDFTLTISSLQPEDFATYYCQQSYSTPLTFGGGTKLEIKRTVAAPSVFIFPPSDEQLKSGTASVVCLLNNFYPREAKVQWKVDNALQSGNSQESVTEQDSKDSTYSLSSTLTLSKADYEKHKVYACEVTHQGLSSPVTKSFNRGEC

SEQ ID NO: 71 - protein, 214 aa, synthetic construct
  source 1..214: note; note (original language) = SL2-5 light chain LC
DIQMTQSPSSLSASVGDRVTITCRASQPISDYLNWYQQKPGKAPKLLIYTASYLESGVPSRFSGSGSGTDFTLTISSLQPEDFATYYCQQSYSTPLTFGGGTKLEIKRTVAAPSVFIFPPSDEQLKSGTASVVCLLNNFYPREAKVQWKVDNALQSGNSQESVTEQDSKDSTYSLSSTLTLSKADYEKHKVYACEVTHQGLSSPVTKSFNRGEC

SEQ ID NO: 72 - protein, 214 aa, synthetic construct
  source 1..214: note = SL2-6 LC
DIQMTQSPSSLSASVGDRVTITCRASQYISDYLNWYQQKPGKAPKLLIYMASALDSGVPSRFSGSGSGTDFTLTISSLQPEDFATYYCQQSYSTPLTFGGGTKLEIKRTVAAPSVFIFPPSDEQLKSGTASVVCLLNNFYPREAKVQWKVDNALQSGNSQESVTEQDSKDSTYSLSSTLTLSKADYEKHKVYACEVTHQGLSSPVTKSFNRGEC

SEQ ID NO: 73 - protein, 214 aa, synthetic construct
  source 1..214: note; note (original language) = SL2-8 light chain LC
DIQMTQSPSSLSASVGDRVTITCRASQYISDYLNWYQQKPGKAPKLLIYAASYLESGVPSRFSGSGSGTDFTLTISSLQPEDFATYYCQQSYSTPLTFGGGTKLEIKRTVAAPSVFIFPPSDEQLKSGTASVVCLLNNFYPREAKVQWKVDNALQSGNSQESVTEQDSKDSTYSLSSTLTLSKADYEKHKVYACEVTHQGLSSPVTKSFNRGEC

SEQ ID NO: 74 - protein, 214 aa, synthetic construct
  source 1..214: note; note (original language) = SL2-9 light chain LC
DIQMTQSPSSLSASVGDRVTITCRASQFISPYLNWYQQKPGKAPKLLIYAASELESGVPSRFSGSGSGTDFTLTISSLQPEDFATYYCQQSYSTPLTFGGGTKLEIKRTVAAPSVFIFPPSDEQLKSGTASVVCLLNNFYPREAKVQWKVDNALQSGNSQESVTEQDSKDSTYSLSSTLTLSKADYEKHKVYACEVTHQGLSSPVTKSFNRGEC

SEQ ID NO: 75 - protein, 214 aa, synthetic construct
  source 1..214: note; note (original language) = SL2-12 light chain LC
DIQMTQSPSSLSASVGDRVTITCRASQYISDYLNWYQQKPGKAPKLLIYSASYLDSGVPSRFSGSGSGTDFTLTISSLQPEDFATYYCQQSYSTPLTFGGGTKLEIKRTVAAPSVFIFPPSDEQLKSGTASVVCLLNNFYPREAKVQWKVDNALQSGNSQESVTEQDSKDSTYSLSSTLTLSKADYEKHKVYACEVTHQGLSSPVTKSFNRGEC

SEQ ID NO: 76 - protein, 214 aa, synthetic construct
  source 1..214: note; note (original language) = SL2-13 light chain LC
DIQMTQSPSSLSASVGDRVTITCRASQVISDYLNWYQQKPGKAPKLLIYAASYLDSGVPSRFSGSGSGTDFTLTISSLQPEDFATYYCQQSYSTPLTFGGGTKLEIKRTVAAPSVFIFPPSDEQLKSGTASVVCLLNNFYPREAKVQWKVDNALQSGNSQESVTEQDSKDSTYSLSSTLTLSKADYEKHKVYACEVTHQGLSSPVTKSFNRGEC

SEQ ID NO: 77 - protein, 214 aa, synthetic construct
  source 1..214: note; note (original language) = SL2-15 light chain LC
DIQMTQSPSSLSASVGDRVTITCRASQKISDYLNWYQQKPGKAPKLLIYAASGLESGVPSRFSGSGSGTDFTLTISSLQPEDFATYYCQQSYSTPLTFGGGTKLEIKRTVAAPSVFIFPPSDEQLKSGTASVVCLLNNFYPREAKVQWKVDNALQSGNSQESVTEQDSKDSTYSLSSTLTLSKADYEKHKVYACEVTHQGLSSPVTKSFNRGEC

SEQ ID NO: 78 - protein, 214 aa, synthetic construct
  source 1..214: note; note (original language) = SL2-17 light chain LC
DIQMTQSPSSLSASVGDRVTITCRASQGISHYLNWYQQKPGKAPKLLIYAASYLDSGVPSRFSGSGSGTDFTLTISSLQPEDFATYYCQQSYSTPLTFGGGTKLEIKRTVAAPSVFIFPPSDEQLKSGTASVVCLLNNFYPREAKVQWKVDNALQSGNSQESVTEQDSKDSTYSLSSTLTLSKADYEKHKVYACEVTHQGLSSPVTKSFNRGEC

SEQ ID NO: 79 - protein, 214 aa, synthetic construct
  source 1..214: note; note (original language) = SL2-18 light chain LC
DIQMTQSPSSLSASVGDRVTITCRASQSISEYLNWYQQKPGKAPKLLIYTASYLESGVPSRFSGSGSGTDFTLTISSLQPEDFATYYCQQSYSTPLTFGGGTKLEIKRTVAAPSVFIFPPSDEQLKSGTASVVCLLNNFYPREAKVQWKVDNALQSGNSQESVTEQDSKDSTYSLSSTLTLSKADYEKHKVYACEVTHQGLSSPVTKSFNRGEC

SEQ ID NO: 80 - protein, 214 aa, synthetic construct
  source 1..214: note; note (original language) = SL2-19 light chain LC
DIQMTQSPSSLSASVGDRVTITCRASQAISPYLNWYQQKPGKAPKLLIYAASELESGVPSRFSGSGSGTDFTLTISSLQPEDFATYYCQQSYSTPLTFGGGTKLEIKRTVAAPSVFIFPPSDEQLKSGTASVVCLLNNFYPREAKVQWKVDNALQSGNSQESVTEQDSKDSTYSLSSTLTLSKADYEKHKVYACEVTHQGLSSPVTKSFNRGEC

SEQ ID NO: 81 - protein, 214 aa, synthetic construct
  source 1..214: note; note (original language) = SL2-22 light chain LC
DIQMTQSPSSLSASVGDRVTITCRASQSISDYLNWYQQKPGKAPKLLIYTASYLDSGVPSRFSGSGSGTDFTLTISSLQPEDFATYYCQQSYSTPLTFGGGTKLEIKRTVAAPSVFIFPPSDEQLKSGTASVVCLLNNFYPREAKVQWKVDNALQSGNSQESVTEQDSKDSTYSLSSTLTLSKADYEKHKVYACEVTHQGLSSPVTKSFNRGEC

SEQ ID NO: 82 - protein, 451 aa, synthetic construct
  source 1..451: note; note (original language) = SL2-22-mIgG2a-FcS antibody heavy chain
EVQLLESGGGLVQPGGSLRLSCAASGFTFSSYAMSWVRQAPGKGLEWVSAISGSGGSTYYADSVKGRFTISRDNSKNTLYLQMNSLRAEDTAVYYCARVDSSGGYWYFDLWGRGTLVTVSSAKTTAPSVYPLAPVCGDTTGSSVTLGCLVKGYFPEPVTLTWNSGSLSSGVHTFPAVLQSDLYTLSSSVTVTSSTWPSQSITCNVAHPASSTKVDKKIEPRGPTIKPCPPCKCPAPNAEGAPSVFIFPPKIKDVLMISLSPIVTCVVVDVSEDDPDVQISWFVNNVEVHTAQTQTHREDYNSTLRVVSALPIQHQDWMSGKEFKCKVNNKQLPSSIERTISKPKGSVRAPQVYVLPPPEEEMTKKQVTLTCMVTDFMPEDIYVEWTNNGKTELNYKNTEPVLDSDGSYFMYSKLRVEKKNWVERNSYSCSVVHEGLHNHHTTKSFSRTPGK

SEQ ID NO: 83 - protein, 214 aa, synthetic construct
  source 1..214: note; note (original language) = SL2-22-mIgG2a-FcS antibody light chain
DIQMTQSPSSLSASVGDRVTITCRASQSISDYLNWYQQKPGKAPKLLIYTASYLDSGVPSRFSGSGSGTDFTLTISSLQPEDFATYYCQQSYSTPLTFGGGTKLEIKRADAAPTVSIFPPSSEQLTSGGASVVCFLNNFYPKDINVKWKIDGSERQNGVLNSWTDQDSKDSTYSMSSTLTLTKDEYERHNSYTCEATHKTSTSPIVKSFNRNEC

SEQ ID NO: 84 - protein, 126 aa, synthetic construct
  source 1..126: note = C19-VHH
QVQLVESGGGSVQAGGSLRLSCTASGFTYCEYDMSWYRQAPGKEREFVSRIASDGRTSYVDSVKGRFTISQDNARNTGYLEMNSLKPEDTAMYYCKTEAVKYSGNWCVAAPGFAYWGQGTQVTVSS

SEQ ID NO: 85 - protein, 5 aa, synthetic construct
  source 1..5: note = CDR1
EYDMS

SEQ ID NO: 86 - protein, 16 aa, synthetic construct
  source 1..16: note = CDR2
RIASDGRTSYVDSVKG

SEQ ID NO: 87 - protein, 18 aa, synthetic construct
  source 1..18: note = CDR3
EAVKYSGNWCVAAPGFAY

SEQ ID NO: 88 - protein, 229 aa, synthetic construct
  source 1..229: note = hIgG4-Fc(S228P)
ESKYGPPCPPCPAPEFLGGPSVFLFPPKPKDTLMISRTPEVTCVVVDVSQEDPEVQFNWYVDGVEVHNAKTKPREEQFNSTYRVVSVLTVLHQDWLNGKEYKCKVSNKGLPSSIEKTISKAKGQPREPQVYTLPPSQEEMTKNQVSLTCLVKGFYPSDIAVEWESNGQPENNYKTTPPVLDSDGSFFLYSRLTVDKSRWQEGNVFSCSVMHEALHNHYTQKSLSLSLGK

SEQ ID NO: 89 - protein, 355 aa, synthetic construct
  source 1..355: note = C19
QVQLVESGGGSVQAGGSLRLSCTASGFTYCEYDMSWYRQAPGKEREFVSRIASDGRTSYVDSVKGRFTISQDNARNTGYLEMNSLKPEDTAMYYCKTEAVKYSGNWCVAAPGFAYWGQGTQVTVSSESKYGPPCPPCPAPEFLGGPSVFLFPPKPKDTLMISRTPEVTCVVVDVSQEDPEVQFNWYVDGVEVHNAKTKPREEQFNSTYRVVSVLTVLHQDWLNGKEYKCKVSNKGLPSSIEKTISKAKGQPREPQVYTLPPSQEEMTKNQVSLTCLVKGFYPSDIAVEWESNGQPENNYKTTPPVLDSDGSFFLYSRLTVDKSRWQEGNVFSCSVMHEALHNHYTQKSLSLSLGK

SEQ ID NO: 90 - protein, 126 aa, synthetic construct
  source 1..126: note = C19-hu3
EVQLLESGGGLVQPGGSLRLSCTASGFTYCEYDMSWYRQAPGKEREFVSRIASDGRTSYVDSVKGRFTISQDNARNTGYLQMNSLRAEDTAVYYCKTEAVKYSGNWCVAAPGFAYWGQGTLVTVSS

SEQ ID NO: 91 - protein, 126 aa, synthetic construct
  source 1..126: note = C19-hu7
EVQLLESGGGLVQPGGSLRLSCTASGFTYCEYDMSWYRQAPGKEREFVSRIASDGRTSYVDSVKGRFTISQDNARNTGYLEMNSLRAEDTAVYYCKTEAVKYSGNWCVAAPGFAYWGQGTLVTVSS

SEQ ID NO: 92 - protein, 126 aa, synthetic construct
  source 1..126: note = C19-hu8
EVQLLESGGGLVQPGGSLRLSCTASGFTYCEYDMSWYRQAPGKEREFVSRIASDGRTSYVDSVKGRFTISQDNSKNTGYLEMNSLRAEDTAVYYCKTEAVKYSGNWCVAAPGFAYWGQGTLVTVSS

SEQ ID NO: 93 - protein, 355 aa, synthetic construct
  source 1..355: note = C19-3
EVQLLESGGGLVQPGGSLRLSCTASGFTYCEYDMSWYRQAPGKEREFVSRIASDGRTSYVDSVKGRFTISQDNARNTGYLQMNSLRAEDTAVYYCKTEAVKYSGNWCVAAPGFAYWGQGTLVTVSSESKYGPPCPPCPAPEFLGGPSVFLFPPKPKDTLMISRTPEVTCVVVDVSQEDPEVQFNWYVDGVEVHNAKTKPREEQFNSTYRVVSVLTVLHQDWLNGKEYKCKVSNKGLPSSIEKTISKAKGQPREPQVYTLPPSQEEMTKNQVSLTCLVKGFYPSDIAVEWESNGQPENNYKTTPPVLDSDGSFFLYSRLTVDKSRWQEGNVFSCSVMHEALHNHYTQKSLSLSLGK

SEQ ID NO: 94 - protein, 355 aa, synthetic construct
  source 1..355: note = C19-7
EVQLLESGGGLVQPGGSLRLSCTASGFTYCEYDMSWYRQAPGKEREFVSRIASDGRTSYVDSVKGRFTISQDNARNTGYLEMNSLRAEDTAVYYCKTEAVKYSGNWCVAAPGFAYWGQGTLVTVSSESKYGPPCPPCPAPEFLGGPSVFLFPPKPKDTLMISRTPEVTCVVVDVSQEDPEVQFNWYVDGVEVHNAKTKPREEQFNSTYRVVSVLTVLHQDWLNGKEYKCKVSNKGLPSSIEKTISKAKGQPREPQVYTLPPSQEEMTKNQVSLTCLVKGFYPSDIAVEWESNGQPENNYKTTPPVLDSDGSFFLYSRLTVDKSRWQEGNVFSCSVMHEALHNHYTQKSLSLSLGK

SEQ ID NO: 95 - protein, 355 aa, synthetic construct
  source 1..355: note = C19-8
EVQLLESGGGLVQPGGSLRLSCTASGFTYCEYDMSWYRQAPGKEREFVSRIASDGRTSYVDSVKGRFTISQDNSKNTGYLEMNSLRAEDTAVYYCKTEAVKYSGNWCVAAPGFAYWGQGTLVTVSSESKYGPPCPPCPAPEFLGGPSVFLFPPKPKDTLMISRTPEVTCVVVDVSQEDPEVQFNWYVDGVEVHNAKTKPREEQFNSTYRVVSVLTVLHQDWLNGKEYKCKVSNKGLPSSIEKTISKAKGQPREPQVYTLPPSQEEMTKNQVSLTCLVKGFYPSDIAVEWESNGQPENNYKTTPPVLDSDGSFFLYSRLTVDKSRWQEGNVFSCSVMHEALHNHYTQKSLSLSLGK

SEQ ID NO: 96 - protein, 8 aa, synthetic construct
  source 1..8: note = CDR1
GFTYCEYD

SEQ ID NO: 97 - protein, 7 aa, synthetic construct
  source 1..7: note = CDR1
GFTYCEY

SEQ ID NO: 98 - protein, 10 aa, synthetic construct
  source 1..10: note = CDR1
GFTYCEYDMS

SEQ ID NO: 99 - protein, 6 aa, synthetic construct
  source 1..6: note = CDR1
CEYDMS

SEQ ID NO: 100 - protein, 608 aa, synthetic construct
  source 1..608: note; note (original language) = Human GARP extracellular domain
HQDKVPCKMVDKKVSCQVLGLLQVPSVLPPDTETLDLSGNQLRSILASPLGFYTALRHLDLSTNEISFLQPGAFQALTHLEHLSLAHNRLAMATALSAGGLGPLPRVTSLDLSGNSLYSGLLERLLGEAPSLHTLSLAENSLTRLTRHTFRDMPALEQLDLHSNVLMDIEDGAFEGLPRLTHLNLSRNSLTCISDFSLQQLRVLDLSCNSIEAFQTASQPQAEFQLTWLDLRENKLLHFPDLAALPRLIYLNLSNNLIRLPTGPPQDSKGIHAPSEGWSALPLSAPSGNASGRPLSQLLNLDLSYNEIELIPDSFLEHLTSLCFLNLSRNCLRTFEARRLGSLPCLMLLDLSHNALETLELGARALGSLRTLLLQGNALRDLPPYTFANLASLQRLNLQGNRVSPCGGPDEPGPSGCVAFSGITSLRSLSLVDNEIELLRAGAFLHTPLTELDLSSNPGLEVATGALGGLEASLEVLALQGNGLMVLQVDLPCFICLKRLNLAENRLSHLPAWTQAVSLEVLDLRNNSFSLLPGSAMGGLETSLRRLYLQGNPLSCCGNGWLAAQLHQGRVDVDATQDLICRFSSQEEVSLSHVRPEDCEKGGLKNIN

SEQ ID NO: 101 - protein, 112 aa, synthetic construct
  source 1..112: note; note (original language) = Mature human TGFβ1
ALDTNYCFSSTEKNCCVRQLYIDFRKDLGWKWIHEPKGYHANFCLGPCPYIWSLDTQYSKVLALYNQHNPGASAAPCCVPQALEPLPIVYYVGRKPKVEQLSNMIVRSCKCS

SEQ ID NO: 102 - protein, 249 aa, synthetic construct
  source 1..249: note; note (original language) = Human LAP
LSTCKTIDMELVKRKRIEAIRGQILSKLRLASPPSQGEVPPGPLPEAVLALYNSTRDRVAGESAEPEPEPEADYYAKEVTRVLMVETHNEIYDKFKQSTHSIYMFFNTSELREAVPEPVLLSRAELRLLRLKLKVEQHVELYQKYSNNSWRYLSNRLLAPSDSPEWLSFDVTGVVRQWLSRGGEIEGFRLSAHCSCDSRDNTLQVDINGFTTGRRGDLATIHGMNRPFLLLMATPLERAQHLQSSRHRR

SEQ ID NO: 103 - protein, 611 aa, synthetic construct
  source 1..611: note; note (original language) = Mouse GARP extracellular domain
ISQRREQVPCRTVNKEALCHGLGLLQVPSVLSLDIQALYLSGNQLQSILVSPLGFYTALRHLDLSDNQISFLQAGVFQALPYLEHLNLAHNRLATGMALNSGGLGRLPLLVSLDLSGNSLHGNLVERLLGETPRLRTLSLAENSLTRLARHTFWGMPAVEQLDLHSNVLMDIEDGAFEALPHLTHLNLSRNSLTCISDFSLQQLQVLDLSCNSIEAFQTAPEPQAQFQLAWLDLRENKLLHFPDLAVFPRLIYLNVSNNLIQLPAGLPRGSEDLHAPSEGWSASPLSNPSRNASTHPLSQLLNLDLSYNEIELVPASFLEHLTSLRFLNLSRNCLRSFEARQVDSLPCLVLLDLSHNVLEALELGTKVLGSLQTLLLQDNALQELPPYTFASLASLQRLNLQGNQVSPCGGPAEPGPPGCVDFSGIPTLHVLNMAGNSMGMLRAGSFLHTPLTELDLSTNPGLDVATGALVGLEASLEVLELQGNGLTVLRVDLPCFLRLKRLNLAENQLSHLPAWTRAVSLEVLDLRNNSFSLLPGNAMGGLETSLRRLYLQGNPLSCCGNGWLAAQLHQGRVDVDATQDLICRFGSQEELSLSLVRPEDCEKGGLKNVN

SEQ ID NO: 104 - protein, 112 aa, synthetic construct
  source 1..112: note; note (original language) = Mature mouse TGFβ1
ALDTNYCFSSTEKNCCVRQLYIDFRKDLGWKWIHEPKGYHANFCLGPCPYIWSLDTQYSKVLALYNQHNPGASASPCCVPQALEPLPIVYYVGRKPKVEQLSNMIVRSCKCS

SEQ ID NO: 105 - protein, 249 aa, synthetic construct
  source 1..249: note; note (original language) = Mouse LAP
LSTCKTIDMELVKRKRIEAIRGQILSKLRLASPPSQGEVPPGPLPEAVLALYNSTRDRVAGESADPEPEPEADYYAKEVTRVLMVDRNNAIYEKTKDISHSIYMFFNTSDIREAVPEPPLLSRAELRLQRLKSSVEQHVELYQKYSNNSWRYLGNRLLTPTDTPEWLSFDVTGVVRQWLNQGDGIQGFRFSAHCSCDSKDNKLHVEINGISPKRRGDLGTIHDMNRPFLLLMATPLERAQHLHSSRHRR

SEQ ID NO: 106 - protein, 355 aa, synthetic construct
  source 1..355: note = C19-8-mIgG2a-FcS
EVQLLESGGGLVQPGGSLRLSCTASGFTYCEYDMSWYRQAPGKEREFVSRIASDGRTSYVDSVKGRFTISQDNSKNTGYLEMNSLRAEDTAVYYCKTEAVKYSGNWCVAAPGFAYWGQGTLVTVSSPTIKPCPPCKCPAPNAEGAPSVFIFPPKIKDVLMISLSPIVTCVVVDVSEDDPDVQISWFVNNVEVHTAQTQTHREDYNSTLRVVSALPIQHQDWMSGKEFKCKVNNKQLPSSIERTISKPKGSVRAPQVYVLPPPEEEMTKKQVTLTCMVTDFMPEDIYVEWTNNGKTELNYKNTEPVLDSDGSYFMYSKLRVEKKNWVERNSYSCSVVHEGLHNHHTTKSFSRTPGK

SEQ ID NO: 107 - protein, 7 aa, synthetic construct
  source 1..7: note = CDR2
IASDGRT

SEQ ID NO: 108 - protein, 5 aa, synthetic construct
  source 1..5: note = CDR2
ASDGR

SEQ ID NO: 109 - protein, 9 aa, synthetic construct
  source 1..9: note = CDR2
RIASDGRTS

SEQ ID NO: 110 - protein, 12 aa, synthetic construct
  source 1..12: note = CDR2
FVSRIASDGRTS

SEQ ID NO: 111 - protein, 20 aa, synthetic construct
  source 1..20: note = CDR3
KTEAVKYSGNWCVAAPGFAY

SEQ ID NO: 112 - protein, 19 aa, synthetic construct
  source 1..19: note = CDR3
KTEAVKYSGNWCVAAPGFA

SEQ ID NO: 113 - protein, 8 aa, synthetic construct
  source 1..8: note = HCDR1
GFTFSSYA

SEQ ID NO: 114 - protein, 7 aa, synthetic construct
  source 1..7: note = HCDR1
GFTFSSY

SEQ ID NO: 115 - protein, 10 aa, synthetic construct
  source 1..10: note = HCDR1
GFTFSSYAMS

SEQ ID NO: 116 - protein, 6 aa, synthetic construct
  source 1..6: note = HCDR1
SSYAMS

SEQ ID NO: 117 - protein, 8 aa, synthetic construct
  source 1..8: note = HCDR2
ISGSGGST

SEQ ID NO: 118 - protein, 6 aa, synthetic construct
  source 1..6: note = HCDR2
SGSGGS

SEQ ID NO: 119 - protein, 10 aa, synthetic construct
  source 1..10: note = HCDR2
AISGSGGSTY

SEQ ID NO: 120 - protein, 13 aa, synthetic construct
  source 1..13: note = HCDR2
WVSAISGSGGSTY

SEQ ID NO: 121 - protein, 14 aa, synthetic construct
  source 1..14: note = HCDR3
ARVDSSGGYWYFDL

SEQ ID NO: 122 - protein, 13 aa, synthetic construct
  source 1..13: note = HCDR3
ARVDSSGGYWYFD

SEQ ID NO: 123 - protein, 6 aa, synthetic construct
  source 1..6: note = LCDR1
QSISDY

SEQ ID NO: 124 - protein, 7 aa, synthetic construct
  source 1..7: note = LCDR1
SDYLNWY

SEQ ID NO: 125 - protein, 10 aa, synthetic construct
  source 1..10: note = LCDR2
LLIYTASYLD

SEQ ID NO: 126 - protein, 8 aa, synthetic construct
  source 1..8: note = LCDR3
QQSYSTPL